European Patent Application EP 4 397 307 A1, published July 10, 2024. Title: Composition for cancer immunotherapy containing STING and TRIM29 interaction inhibitor as an active ingredient. Applicant: SNU R&DB Foundation. Application KR. The sequence listing filed with the application follows.

SEQUENCE LISTING (10 sequences)

SEQ ID NO: 1 - DNA, 20 bp, synthetic construct
  misc_feature 1..20: note = mGAPDH_F primer
  source 1..20: mol_type = other DNA
tgggctacactgagcaccag

SEQ ID NO: 2 - DNA, 20 bp, synthetic construct
  misc_feature 1..20: note = mGAPDH_R primer
  source 1..20: mol_type = other DNA
gggtgtcgctgttgaagtca

SEQ ID NO: 3 - DNA, 24 bp, synthetic construct
  misc_feature 1..24: note = mIFNbeta_F primer
  source 1..24: mol_type = other DNA
aagagttacactgcctttgccatc

SEQ ID NO: 4 - DNA, 24 bp, synthetic construct
  misc_feature 1..24: note = mIFNbeta_R primer
  source 1..24: mol_type = other DNA
cactgtctgctggtggagttcatc

SEQ ID NO: 5 - DNA, 20 bp, synthetic construct
  misc_feature 1..20: note = mIL6_F primer
  source 1..20: mol_type = other DNA
tccagttgccttcttgggac

SEQ ID NO: 6 - DNA, 20 bp, synthetic construct
  misc_feature 1..20: note = mIL6_R primer
  source 1..20: mol_type = other DNA
gtactccagaagaccagagg

SEQ ID NO: 7 - DNA, 20 bp, synthetic construct
  misc_feature 1..20: note = mIL15_F primer
  source 1..20: mol_type = other DNA
gtgactttcatcccagttgc

SEQ ID NO: 8 - DNA, 20 bp, synthetic construct
  misc_feature 1..20: note = mIL15_R primer
  source 1..20: mol_type = other DNA
ttccttgcagccagattctg

SEQ ID NO: 9 - DNA, 21 bp, synthetic construct
  misc_feature 1..21: note = mIL15Ralpha_F primer
  source 1..21: mol_type = other DNA
cccacagttccaaaatgacga

SEQ ID NO: 10 - DNA, 23 bp, synthetic construct
  misc_feature 1..23: note = mIL15Ralpha_R primer
  source 1..23: mol_type = other DNA
gctgccttgatttgatgtaccag